European Patent Application EP 4 450 520 A1, published October 23, 2024. Title: PD-L1 ANTIGEN BINDING PROTEIN AND APPLICATION THEREOF. Applicant: SHANGHAI HUAOTA BIOPHARMACEUTICAL CO., LTD. The sequence listing filed with the application follows.

SEQUENCE LISTING (57 sequences)

SEQ ID NO: 1 - protein, 5 aa, synthetic construct
  REGION 1..5: note = HCDR1
DYYIN

SEQ ID NO: 2 - protein, 17 aa, synthetic construct
  REGION 1..17: note = HCDR2
WIYLGSGNAKYNEKFKG

SEQ ID NO: 3 - protein, 10 aa, synthetic construct
  REGION 1..10: note = HCDR3
CVGTYWYFDV

SEQ ID NO: 4 - protein, 17 aa, synthetic construct
  REGION 1..17: note = HCDR2 3; 5
WIYLGSGNAKYSQKFQG

SEQ ID NO: 5 - protein, 10 aa, synthetic construct
  REGION 1..10: note = HCDR3 4; 5
SVGTYWYFDV

SEQ ID NO: 6 - protein, 10 aa, synthetic construct
  REGION 1..10: note = LCDR1
SASSSVSYMH

SEQ ID NO: 7 - protein, 7 aa, synthetic construct
  REGION 1..7: note = LCDR2
DTSNVAS

SEQ ID NO: 8 - protein, 9 aa, synthetic construct
  REGION 1..9: note = LCDR3
HQRSSYPWT

SEQ ID NO: 9 - protein, 7 aa, synthetic construct
  REGION 1..7: note = LCDR2 2
DTSNVQS

SEQ ID NO: 10 - protein, 7 aa, synthetic construct
  REGION 1..7: note = LCDR2 3
DTSSLQS

SEQ ID NO: 11 - protein, 119 aa, synthetic construct
  REGION 1..119: note = VH
QIQLQQSGPELVKPGASVKISCKASGYTFTDYYINWVKQRPGQGLEWIGWIYLGSGNAKYNEKFKGKATLTVDTSSSTAYMHLSSLTSEDSAVYFCARCVGTYWYFDVWGAGTTVTVSS

SEQ ID NO: 12 - protein, 119 aa, synthetic construct
  REGION 1..119: note = huVH1
QIQLVQSGAEVKKPGASVKISCKASGYTFTDYYINWVRQAPGQRLEWIGWIYLGSGNAKYNEKFKGKATLTVDTSASTAYMELSSLRSEDTAVYFCARCVGTYWYFDVWGQGTTVTVSS

SEQ ID NO: 13 - protein, 119 aa, synthetic construct
  REGION 1..119: note = huVH2
QIQLVQSGAEVKKPGASVKVSCKASGYTFTDYYINWVRQAPGQRLEWIGWIYLGSGNAKYNEKFKGRATLTVDTSASTAYMELSSLRSEDTAVYYCARCVGTYWYFDVWGQGTTVTVSS

SEQ ID NO: 14 - protein, 119 aa, synthetic construct
  REGION 1..119: note = huVH3
QIQLVQSGAEVKKPGASVKVSCKASGYTFTDYYINWVRQAPGQRLEWIGWIYLGSGNAKYSQKFQGRATLTVDTSASTAYMELSSLRSEDTAVYYCARCVGTYWYFDVWGQGTTVTVSS

SEQ ID NO: 15 - protein, 119 aa, synthetic construct
  REGION 1..119: note = huVH4
QVQLVQSGAEVKKPGASVKVSCKASGYTFTDYYINWVRQAPGQRLEWIGWIYLGSGNAKYNEKFKGRVTITVDTSASTAYMELSSLRSEDTAVYYCARSVGTYWYFDVWGQGTTVTVSS

SEQ ID NO: 16 - protein, 119 aa, synthetic construct
  REGION 1..119: note = huVH5
QVQLVQSGAEVKKPGASVKVSCKASGYTFTDYYINWVRQAPGQRLEWIGWIYLGSGNAKYSQKFQGRVTITVDTSASTAYMELSSLRSEDTAVYYCARSVGTYWYFDVWGQGTTVTVSS

SEQ ID NO: 17 - protein, 106 aa, synthetic construct
  REGION 1..106: note = VL
QILLTQSPATMSASPGEKVTMTCSASSSVSYMHWYQQKPGSSPKPWIYDTSNVASGFPARFSGSGSGTSYSLIISSMEAEDAATYYCHQRSSYPWTFGGGTKLEIK

SEQ ID NO: 18 - protein, 106 aa, synthetic construct
  REGION 1..106: note = huVL1
QIQLTQSPSSLSASVGDRVTMTCSASSSVSYMHWYQQKPGKAPKPWIYDTSNVASGFPARFSGSGSGTDYTLTISSMQPEDFATYYCHQRSSYPWTFGQGTKLEIK

SEQ ID NO: 19 - protein, 106 aa, synthetic construct
  REGION 1..106: note = huVL2
DIQLTQSPSSLSASVGDRVTITCSASSSVSYMHWYQQKPGKAPKPWIYDTSNVQSGFPSRFSGSGSGTDYTLTISSLQPEDFATYYCHQRSSYPWTFGQGTKLEIK

SEQ ID NO: 20 - protein, 106 aa, synthetic construct
  REGION 1..106: note = huVL3
DIQLTQSPSSLSASVGDRVTITCSASSSVSYMHWYQQKPGKAPKLLIYDTSSLQSGVPSRFSGSGSGTDYTLTISSLQPEDFATYYCHQRSSYPWTFGQGTKLEIK

SEQ ID NO: 21 - protein, 17 aa, synthetic construct
  REGION 1..17: note = HCDR2; HCDR2 3; 5
  SITE 12: note = misc_feature - Xaa = Asn or Ser
  SITE 13: note = misc_feature - Xaa = Glu or Gln
  SITE 16: note = misc_feature - Xaa = Lys or Gln
WIYLGSGNAKYXXKFXG

SEQ ID NO: 22 - protein, 10 aa, synthetic construct
  REGION 1..10: note = HCDR3; HCDR3 4; 5
  SITE 1: note = misc_feature - Xaa = Cys or Ser
XVGTYWYFDV

SEQ ID NO: 23 - protein, 7 aa, synthetic construct
  REGION 1..7: note = LCDR2; LCDR22; LCDR23
  SITE 4: note = misc_feature - Xaa = Asn or Ser
  SITE 5: note = misc_feature - Xaa = Leu or Val
  SITE 6: note = misc_feature - Xaa = Ala or Gln
DTSXXXS

SEQ ID NO: 24 - protein, 30 aa, synthetic construct
  REGION 1..30: note = HFR1-245
QIQLQQSGPELVKPGASVKISCKASGYTFT

SEQ ID NO: 25 - protein, 30 aa, synthetic construct
  REGION 1..30: note = HFR1-1
QIQLVQSGAEVKKPGASVKISCKASGYTFT

SEQ ID NO: 26 - protein, 30 aa, synthetic construct
  REGION 1..30: note = HFR1-2; 3
QIQLVQSGAEVKKPGASVKVSCKASGYTFT

SEQ ID NO: 27 - protein, 30 aa, synthetic construct
  REGION 1..30: note = HFR1-4; 5
QVQLVQSGAEVKKPGASVKVSCKASGYTFT

SEQ ID NO: 28 - protein, 14 aa, synthetic construct
  REGION 1..14: note = HFR2-245
WVKQRPGQGLEWIG

SEQ ID NO: 29 - protein, 14 aa, synthetic construct
  REGION 1..14: note = HFR2-1; 2; 3; 4; 5
WVRQAPGQRLEWIG

SEQ ID NO: 30 - protein, 32 aa, synthetic construct
  REGION 1..32: note = HFR3-245
KATLTVDTSSSTAYMHLSSLTSEDSAVYFCAR

SEQ ID NO: 31 - protein, 32 aa, synthetic construct
  REGION 1..32: note = HFR3-1
KATLTVDTSASTAYMELSSLRSEDTAVYFCAR

SEQ ID NO: 32 - protein, 32 aa, synthetic construct
  REGION 1..32: note = HFR3-2; 3
RATLTVDTSASTAYMELSSLRSEDTAVYYCAR

SEQ ID NO: 33 - protein, 32 aa, synthetic construct
  REGION 1..32: note = HFR3-4; 5
RVTITVDTSASTAYMELSSLRSEDTAVYYCAR

SEQ ID NO: 34 - protein, 11 aa, synthetic construct
  REGION 1..11: note = HFR4-245
WGAGTTVTVSS

SEQ ID NO: 35 - protein, 11 aa, synthetic construct
  REGION 1..11: note = HFR4-1; 2; 3; 4; 5
WGQGTTVTVSS

SEQ ID NO: 36 - protein, 23 aa, synthetic construct
  REGION 1..23: note = LFR1-245
QILLTQSPATMSASPGEKVTMTC

SEQ ID NO: 37 - protein, 22 aa, synthetic construct
  REGION 1..22: note = LFR1-1
QIQLTQSPSSLSASVGDRVTMT

SEQ ID NO: 38 - protein, 23 aa, synthetic construct
  REGION 1..23: note = LFR1-2; 3
DIQLTQSPSSLSASVGDRVTITC

SEQ ID NO: 39 - protein, 15 aa, synthetic construct
  REGION 1..15: note = LFR2-245
WYQQKPGSSPKPWIY

SEQ ID NO: 40 - protein, 15 aa, synthetic construct
  REGION 1..15: note = LFR2-1; 2
WYQQKPGKAPKPWIY

SEQ ID NO: 41 - protein, 15 aa, synthetic construct
  REGION 1..15: note = LFR2-3
WYQQKPGKAPKLLIY

SEQ ID NO: 42 - protein, 32 aa, synthetic construct
  REGION 1..32: note = LFR3-245
GFPARFSGSGSGTSYSLIISSMEAEDAATYYC

SEQ ID NO: 43 - protein, 32 aa, synthetic construct
  REGION 1..32: note = LFR3-1
GFPARFSGSGSGTDYTLTISSMQPEDFATYYC

SEQ ID NO: 44 - protein, 32 aa, synthetic construct
  REGION 1..32: note = LFR3-2
GFPSRFSGSGSGTDYTLTISSLQPEDFATYYC

SEQ ID NO: 45 - protein, 32 aa, synthetic construct
  REGION 1..32: note = LFR3-3
GVPSRFSGSGSGTDYTLTISSLQPEDFATYYC

SEQ ID NO: 46 - protein, 10 aa, synthetic construct
  REGION 1..10: note = LFR4-245
FGGGTKLEIK

SEQ ID NO: 47 - protein, 10 aa, synthetic construct
  REGION 1..10: note = LFR4-1; 2; 3
FGQGTKLEIK

SEQ ID NO: 48 - protein, 30 aa, synthetic construct
  REGION 1..30: note = HFR1 general formula
  SITE 2: note = misc_feature - Xaa = Ile or Val
  SITE 5: note = misc_feature - Xaa = Gln or Val
  SITE 9: note = misc_feature - Xaa = Ala or Pro
  SITE 11: note = misc_feature - Xaa = Leu or Val
  SITE 12: note = misc_feature - Xaa = Lys or Val
  SITE 20: note = misc_feature - Xaa = Ile or Val
QXQLXQSGXEXXKPGASVKXSCKASGYTFT

SEQ ID NO: 49 - protein, 14 aa, synthetic construct
  REGION 1..14: note = HFR2 general formula
  SITE 3: note = misc_feature - Xaa = Lys or Arg
  SITE 5: note = misc_feature - Xaa = Ala or Arg
  SITE 9: note = misc_feature - Xaa = Gly or Arg
WVXQXPGQXLEWIG

SEQ ID NO: 50 - protein, 32 aa, synthetic construct
  REGION 1..32: note = HFR3 general formula
  SITE 1: note = misc_feature - Xaa = Lys or Arg
  SITE 2: note = misc_feature - Xaa = Ala or Val
  SITE 4: note = misc_feature - Xaa = Ile or Leu
  SITE 10: note = misc_feature - Xaa = Ala or Ser
  SITE 16: note = misc_feature - Xaa = Glu or His
  SITE 21: note = misc_feature - Xaa = Arg or Thr
  SITE 25: note = misc_feature - Xaa = Ser or Thr
  SITE 29: note = misc_feature - Xaa = Phe or Tyr
XXTXTVDTSXSTAYMXLSSLXSEDXAVYXCAR

SEQ ID NO: 51 - protein, 15 aa, synthetic construct
  REGION 1..15: note = LFR2 general formula
  SITE 8: note = misc_feature - Xaa = Lys or Ser
  SITE 9: note = misc_feature - Xaa = Ala or Ser
  SITE 12: note = misc_feature - Xaa = Leu or Pro
  SITE 13: note = misc_feature - Xaa = Leu or Trp
WYQQKPGXXPKXXIY

SEQ ID NO: 52 - protein, 32 aa, synthetic construct
  REGION 1..32: note = LFR3 general formula
  SITE 2: note = misc_feature - Xaa = Phe or Val
  SITE 4: note = misc_feature - Xaa = Ala or Ser
  SITE 14: note = misc_feature - Xaa = Asp or Ser
  SITE 16: note = misc_feature - Xaa = Ser or Thr
  SITE 18: note = misc_feature - Xaa = Ile or Thr
  SITE 22: note = misc_feature - Xaa = Leu or Met
  SITE 23: note = misc_feature - Xaa = Glu or Gln
  SITE 24: note = misc_feature - Xaa = Ala or Pro
  SITE 27: note = misc_feature - Xaa = Ala or Phe
GXPXRFSGSGSGTXYXLXISSXXXEDXATYYC

SEQ ID NO: 53 - protein, 10 aa, synthetic construct
  REGION 1..10: note = LFR4 general formula
  SITE 3: note = misc_feature - Xaa = Gly or Gln
FGXGTKLEIK

SEQ ID NO: 54 - protein, 11 aa, synthetic construct
  REGION 1..11: note = HFR4-245; HFR4-1; 2; 3; 4; 5
  SITE 3: note = misc_feature - Xaa = Ala or Gln
WGXGTTVTVSS

SEQ ID NO: 55 - protein, 329 aa, synthetic construct
  REGION 1..329: note = human IgG1 constant region
ASTKGPSVFPLAPSSKSTSGGTAALGCLVKDYFPEPVTVSWNSGALTSGVHTFPAVLQSSGLYSLSSVVTVPSSSLGTQTYICNVNHKPSNTKVDKRVEPKSCDKTHTCPPCPAPEAAGGPSVFLFPPKPKDTLMISRTPEVTCVVVDVSHEDPEVKFNWYVDGVEVHNAKTKPREEQYNSTYRVVSVLTVLHQDWLNGKEYKCKVSNKALPAPIEKTISKAKGQPREPQVYTLPPSREEMTKNQVSLTCLVKGFYPSDIAVEWESNGQPENNYKTTPPVLDSDGSFFLYSKLTVDKSRWQQGNVFSCSVMHEALHNHYTQKSLSLSPG

SEQ ID NO: 56 - protein, 107 aa, synthetic construct [sequence omitted]

SEQ ID NO: 57 - protein, 456 aa, synthetic construct
  REGION 1..456: note = human PD-L1-moFc recombinant protein
FTVTVPKDLYVVEYGSNMTIECKFPVEKQLDLAALIVYWEMEDKNIIQFVHGEEDLKVQHSSYRQRARLLKDQLSLGNAALQITDVKLQDAGVYRCMISYGGADYKRITVKVNAPYNKINQRILVVDPVTSEHELTCQAEGYPKAEVIWTSSDHQVLSGKTTTTNSKREEKLFNVTSTLRINTTTNEIFYCTFRRLDPEENHTAELVIPELPLAHPPNERGGGSEPRGPTIKPCPPCKCPAPNLLGGPSVFIFPPKIKDVLMISLSPIVTCVVVDVSEDDPDVQISWFVNNVEVHTAQTQTHREDYNSTLRVVSALPIQHQDWMSGKEFKCKVNNKDLPAPIERTISKPKGSVRAPQVYVLPPPEEEMTKKQVTLTCMVTDFMPEDIYVEWTNNGKTELNYKNTEPVLDSDGSYFMYSKLRVEKKNWVERNSYSCSVVHEGLHNHHTTKSFSRTPG